European Patent Specification EP 3 720 268 B1, published February 26, 2025. Title: Stevia Cultivar '16228013'. Applicant: PureCircle USA Inc. Application 62/595,609. The sequence listing filed with the application follows.

SEQUENCE LISTING (6 sequences)

SEQ ID NO: 1 - DNA, 102 bp, Stevia rebaudiana
  variation (56)..(56): Where "R" is either "G" or "A"
aaaaatagactttttaccatctcttcctctcaagtctcaatctcaacacctacacrtgtatgttttttcaaacaaaccacacacattggttttgatctaaaa

SEQ ID NO: 2 - DNA, 102 bp, Stevia rebaudiana
  variation (61)..(61): Where "Y" is either "C" or "T"
ggtaataacaaccttagttgcctaattatatatgcttcttgtgatgaatttccaatctaaytgtacttgagctaatatagaaaacctagttgctgccacatt

SEQ ID NO: 3 - DNA, 95 bp, Stevia rebaudiana
  variation (52)..(52): Where "S" is either "G" or "C"
gattggtaattggaagtgttgtttattacatatggcaagagaggaaccttasattgtttcaaggtaagtctcgtggttatgatgatgtgtgcaag

SEQ ID NO: 4 - DNA, 98 bp, Stevia rebaudiana
  variation (49)..(49): Where "Y" is either "T" or "C"
aaaatggaaacattttctttttacatttcagcatctgagttgactcggytgcaatcacaaatatgtggaaaaaatggtgatcaccaagttccagagtt

SEQ ID NO: 5 - DNA, 103 bp, Stevia rebaudiana
  variation (49)..(49): Where "W" is either "A" or "T"
atggaagatgaacctgatgttcctgaacaactcgttcgccgatcggttwgtctcgaaatccattcacaagttcttttatattgcactgatttgatacttaggg

SEQ ID NO: 6 - DNA, 101 bp, Stevia rebaudiana
  variation (48)..(48): Where "Y" is either "C" or "T"
agaagaacagtgccagaataatctgtggcgctaaagtgatccaaccayacccttgttctcccagttatataaaagattaaaaattgctagttgtccttcgc